European Patent Application EP 4 386 763 A2, published June 19, 2024. Title: COMPUTER FILES AND METHODS SUPPORTING FORENSIC ANALYSIS OF NUCLEOTIDE SEQUENCE DATA. Applicant: BATTELLE MEMORIAL INSTITUTE. Application EP. The sequence listing filed with the application follows.

SEQUENCE LISTING (52 sequences)

SEQ ID NO: 1 - DNA, 35 bp, Homo sapiens
  source 1..35: mol_type = unassigned DNA
aatgaatgaatgaatgaatgatgaatgaatgaatg

SEQ ID NO: 2 - DNA, 83 bp, unidentified
  misc_feature 1..83: note = Description of Unidentified: Illustrative oligonucleotide
  source 1..83: mol_type = unassigned DNA
gcagacccataatgtcaatagatgtggtagaagtcgtcatttggcgagaaagctcagtcccaggaggaagcggagcagtccaa

SEQ ID NO: 3 - DNA, 83 bp, unidentified
  misc_feature 1..83: note = Description of Unidentified: Illustrative oligonucleotide
  source 1..83: mol_type = unassigned DNA
ttccaatcatagccacagtttacaacatttgtatctttatctgtatccttatttatacatctatctatctatctatctatcta

SEQ ID NO: 4 - DNA, 83 bp, unidentified
  misc_feature 1..83: note = Description of Unidentified: Illustrative oligonucleotide
  source 1..83: mol_type = unassigned DNA
cttcctactggcccataatccagctgtgggagggagccagtggatttggaaaccgacatggcttggccttgcctgcctgcctc

SEQ ID NO: 5 - DNA, 157 bp, unidentified
  misc_feature 1..157: note = Description of Unidentified: Illustrative polynucleotide
  source 1..157: mol_type = unassigned DNA
ccagggcagtgttccaacctgagtctgccaaggcctagcaggttgctaaccaccctgtgtctcagttttcctacctgtaaaatgaagatattaccagtaactgccttcatagatagaagatagatagattagatggatagatagatagatagataga

SEQ ID NO: 6 - DNA, 157 bp, unidentified
  misc_feature 1..157: note = Description of Unidentified: Illustrative polynucleotide
  source 1..157: mol_type = unassigned DNA
ccagggcagtgttccaacctgagtctgccaaggactagcaggttgctaaccaccctgtgtctcagttttcctacctgtaaaatgaagatattaacagtaactgccttcatagatagaagatagatagattagatagttagatagatagatagataga

SEQ ID NO: 7 - DNA, 157 bp, unidentified
  misc_feature 1..157: note = Description of Unidentified: Illustrative polynucleotide
  source 1..157: mol_type = unassigned DNA
ccagggcagtgttccaacctgagtctgccaaggactagcaggttgctaaccaccctgtgtctcagttttcctacctgtaaaatgaagatattaacagtaactgccttcatagatagaagatagatagattagatagatagatagatagatagataga

SEQ ID NO: 8 - DNA, 40 bp, unidentified
  misc_feature 1..40: note = Description of Unidentified: Illustrative oligonucleotide
  source 1..40: mol_type = unassigned DNA
agatagatagatagatagatagatagatagatagatagat

SEQ ID NO: 9 - DNA, 52 bp, unidentified
  misc_feature 1..52: note = Description of Unidentified: Illustrative oligonucleotide
  source 1..52: mol_type = unassigned DNA
agatagatagatagatagatagatagatagatagatagatagatagatagat

SEQ ID NO: 10 - DNA, 48 bp, unidentified
  misc_feature 1..48: note = Description of Unidentified: Illustrative oligonucleotide
  source 1..48: mol_type = unassigned DNA
agatagatagatagatagatagatagatagatagatagatagatagat

SEQ ID NO: 11 - DNA, 36 bp, unidentified
  misc_feature 1..36: note = Description of Unidentified: Illustrative oligonucleotide
  source 1..36: mol_type = unassigned DNA
agatagatagatagatagatagatagatagatagat

SEQ ID NO: 12 - DNA, 20 bp, unidentified
  misc_feature 1..20: note = Description of Unidentified: Illustrative oligonucleotide
  source 1..20: mol_type = unassigned DNA
agatagatagatagatagat

SEQ ID NO: 13 - DNA, 107 bp, unidentified
  misc_feature 1..107: note = Description of Unidentified: Illustrative polynucleotide
  source 1..107: mol_type = unassigned DNA
tctatctatctatctatctgtctgtctgtctgtctgtctgtctatctatctatatctatctatctatcatctatctatccatatctatctatctatctatctatcta

SEQ ID NO: 14 - DNA, 12 bp, unidentified
  misc_feature 1..12: note = Description of Unidentified: Illustrative oligonucleotide
  source 1..12: mol_type = unassigned DNA
tctatctatcta

SEQ ID NO: 15 - DNA, 16 bp, unidentified
  misc_feature 1..16: note = Description of Unidentified: Illustrative oligonucleotide
  source 1..16: mol_type = unassigned DNA
tctatctatctatcta

SEQ ID NO: 16 - DNA, 20 bp, unidentified
  misc_feature 1..20: note = Description of Unidentified: Illustrative oligonucleotide
  source 1..20: mol_type = unassigned DNA
tctatctatctatctatctg

SEQ ID NO: 17 - DNA, 24 bp, unidentified
  misc_feature 1..24: note = Description of Unidentified: Illustrative oligonucleotide
  source 1..24: mol_type = unassigned DNA
tctatctatctatctatctgtctg

SEQ ID NO: 18 - DNA, 28 bp, unidentified
  misc_feature 1..28: note = Description of Unidentified: Illustrative oligonucleotide
  source 1..28: mol_type = unassigned DNA
tctatctatctatctatctgtctgtctg

SEQ ID NO: 19 - DNA, 32 bp, unidentified
  misc_feature 1..32: note = Description of Unidentified: Illustrative oligonucleotide
  source 1..32: mol_type = unassigned DNA
tctatctatctatctatctgtctgtctgtctg

SEQ ID NO: 20 - DNA, 36 bp, unidentified
  misc_feature 1..36: note = Description of Unidentified: Illustrative oligonucleotide
  source 1..36: mol_type = unassigned DNA
tctatctatctatctatctgtctgtctgtctgtctg

SEQ ID NO: 21 - DNA, 40 bp, unidentified
  misc_feature 1..40: note = Description of Unidentified: Illustrative oligonucleotide
  source 1..40: mol_type = unassigned DNA
tctatctatctatctatctgtctgtctgtctgtctgtctg

SEQ ID NO: 22 - DNA, 44 bp, unidentified
  misc_feature 1..44: note = Description of Unidentified: Illustrative oligonucleotide
  source 1..44: mol_type = unassigned DNA
tctatctatctatctatctgtctgtctgtctgtctgtctgtcta

SEQ ID NO: 23 - DNA, 48 bp, unidentified
  misc_feature 1..48: note = Description of Unidentified: Illustrative oligonucleotide
  source 1..48: mol_type = unassigned DNA
tctatctatctatctatctgtctgtctgtctgtctgtctgtctatcta

SEQ ID NO: 24 - DNA, 52 bp, unidentified
  misc_feature 1..52: note = Description of Unidentified: Illustrative oligonucleotide
  source 1..52: mol_type = unassigned DNA
tctatctatctatctatctgtctgtctgtctgtctgtctgtctatctatcta

SEQ ID NO: 25 - DNA, 53 bp, unidentified
  misc_feature 1..53: note = Description of Unidentified: Illustrative oligonucleotide
  source 1..53: mol_type = unassigned DNA
tctatctatctatctatctgtctgtctgtctgtctgtctgtctatctatctat

SEQ ID NO: 26 - DNA, 54 bp, unidentified
  misc_feature 1..54: note = Description of Unidentified: Illustrative oligonucleotide
  source 1..54: mol_type = unassigned DNA
tctatctatctatctatctgtctgtctgtctgtctgtctgtctatctatctata

SEQ ID NO: 27 - DNA, 58 bp, unidentified
  misc_feature 1..58: note = Description of Unidentified: Illustrative oligonucleotide
  source 1..58: mol_type = unassigned DNA
tctatctatctatctatctgtctgtctgtctgtctgtctgtctatctatctatatcta

SEQ ID NO: 28 - DNA, 62 bp, unidentified
  misc_feature 1..62: note = Description of Unidentified: Illustrative oligonucleotide
  source 1..62: mol_type = unassigned DNA
tctatctatctatctatctgtctgtctgtctgtctgtctgtctatctatctatatctatcta

SEQ ID NO: 29 - DNA, 66 bp, unidentified
  misc_feature 1..66: note = Description of Unidentified: Illustrative oligonucleotide
  source 1..66: mol_type = unassigned DNA
tctatctatctatctatctgtctgtctgtctgtctgtctgtctatctatctatatctatctatcta

SEQ ID NO: 30 - DNA, 67 bp, unidentified
  misc_feature 1..67: note = Description of Unidentified: Illustrative oligonucleotide
  source 1..67: mol_type = unassigned DNA
tctatctatctatctatctgtctgtctgtctgtctgtctgtctatctatctatatctatctatctat

SEQ ID NO: 31 - DNA, 68 bp, unidentified
  misc_feature 1..68: note = Description of Unidentified: Illustrative oligonucleotide
  source 1..68: mol_type = unassigned DNA
tctatctatctatctatctgtctgtctgtctgtctgtctgtctatctatctatatctatctatctatc

SEQ ID NO: 32 - DNA, 69 bp, unidentified
  misc_feature 1..69: note = Description of Unidentified: Illustrative oligonucleotide
  source 1..69: mol_type = unassigned DNA
tctatctatctatctatctgtctgtctgtctgtctgtctgtctatctatctatatctatctatctatca

SEQ ID NO: 33 - DNA, 73 bp, unidentified
  misc_feature 1..73: note = Description of Unidentified: Illustrative oligonucleotide
  source 1..73: mol_type = unassigned DNA
tctatctatctatctatctgtctgtctgtctgtctgtctgtctatctatctatatctatctatctatcatcta

SEQ ID NO: 34 - DNA, 77 bp, unidentified
  misc_feature 1..77: note = Description of Unidentified: Illustrative oligonucleotide
  source 1..77: mol_type = unassigned DNA
tctatctatctatctatctgtctgtctgtctgtctgtctgtctatctatctatatctatctatctatcatctatcta

SEQ ID NO: 35 - DNA, 81 bp, unidentified
  misc_feature 1..81: note = Description of Unidentified: Illustrative oligonucleotide
  source 1..81: mol_type = unassigned DNA
tctatctatctatctatctgtctgtctgtctgtctgtctgtctatctatctatatctatctatctatcatctatctatcca

SEQ ID NO: 36 - DNA, 82 bp, unidentified
  misc_feature 1..82: note = Description of Unidentified: Illustrative oligonucleotide
  source 1..82: mol_type = unassigned DNA
tctatctatctatctatctgtctgtctgtctgtctgtctgtctatctatctatatctatctatctatcatctatctatccat

SEQ ID NO: 37 - DNA, 83 bp, unidentified
  misc_feature 1..83: note = Description of Unidentified: Illustrative oligonucleotide
  source 1..83: mol_type = unassigned DNA
tctatctatctatctatctgtctgtctgtctgtctgtctgtctatctatctatatctatctatctatcatctatctatccata

SEQ ID NO: 38 - DNA, 87 bp, unidentified
  misc_feature 1..87: note = Description of Unidentified: Illustrative oligonucleotide
  source 1..87: mol_type = unassigned DNA
tctatctatctatctatctgtctgtctgtctgtctgtctgtctatctatctatatctatctatctatcatctatctatccatatcta

SEQ ID NO: 39 - DNA, 91 bp, unidentified
  misc_feature 1..91: note = Description of Unidentified: Illustrative oligonucleotide
  source 1..91: mol_type = unassigned DNA
tctatctatctatctatctgtctgtctgtctgtctgtctgtctatctatctatatctatctatctatcatctatctatccatatctatcta

SEQ ID NO: 40 - DNA, 95 bp, unidentified
  misc_feature 1..95: note = Description of Unidentified: Illustrative oligonucleotide
  source 1..95: mol_type = unassigned DNA
tctatctatctatctatctgtctgtctgtctgtctgtctgtctatctatctatatctatctatctatcatctatctatccatatctatctatcta

SEQ ID NO: 41 - DNA, 99 bp, unidentified
  misc_feature 1..99: note = Description of Unidentified: Illustrative oligonucleotide
  source 1..99: mol_type = unassigned DNA
tctatctatctatctatctgtctgtctgtctgtctgtctgtctatctatctatatctatctatctatcatctatctatccatatctatctatctatcta

SEQ ID NO: 42 - DNA, 103 bp, unidentified
  misc_feature 1..103: note = Description of Unidentified: Illustrative polynucleotide
  source 1..103: mol_type = unassigned DNA
tctatctatctatctatctgtctgtctgtctgtctgtctgtctatctatctatatctatctatctatcatctatctatccatatctatctatctatctatcta

SEQ ID NO: 43 - DNA, 60 bp, unidentified
  misc_feature 1..60: note = Description of Unidentified: Illustrative oligonucleotide
  source 1..60: mol_type = unassigned DNA
tttctttctttcttttttctctttctttctttctttctttctttctttctccttccttcc

SEQ ID NO: 44 - DNA, 64 bp, unidentified
  misc_feature 1..64: note = Description of Unidentified: Illustrative oligonucleotide
  source 1..64: mol_type = unassigned DNA
tttctttctttcttttttctctttctttctttctttctttctttctttctttctccttccttcc

SEQ ID NO: 45 - DNA, 65 bp, unidentified
  misc_feature 1..65: note = Description of Unidentified: Illustrative oligonucleotide
  source 1..65: mol_type = unassigned DNA
tttctttctttcttttttctctttctttctttctttcttttctttctttctttctccttccttcc

SEQ ID NO: 46 - DNA, 66 bp, unidentified
  misc_feature 1..66: note = Description of Unidentified: Illustrative oligonucleotide
  source 1..66: mol_type = unassigned DNA
tttctttctttcttttttctttctttctttctttctttctttctttctttctttctccttccttcc

SEQ ID NO: 47 - DNA, 68 bp, unidentified
  misc_feature 1..68: note = Description of Unidentified: Illustrative oligonucleotide
  source 1..68: mol_type = unassigned DNA
tttctttctttcttttttctctttctttctttctttctttctttctttctttctttctccttccttcc

SEQ ID NO: 48 - DNA, 72 bp, unidentified
  misc_feature 1..72: note = Description of Unidentified: Illustrative oligonucleotide
  source 1..72: mol_type = unassigned DNA
tttctttctttcttttttctctttctttctttctttctttctttctttctttctttctttctccttccttcc

SEQ ID NO: 49 - DNA, 74 bp, unidentified
  misc_feature 1..74: note = Description of Unidentified: Illustrative oligonucleotide
  source 1..74: mol_type = unassigned DNA
tttctttctttcttttttctttctttctttctttctttctttctttctttctttctttctttctccttccttcc

SEQ ID NO: 50 - DNA, 76 bp, unidentified
  misc_feature 1..76: note = Description of Unidentified: Illustrative oligonucleotide
  source 1..76: mol_type = unassigned DNA
tttctttctttcttttttctctttctttctttctttctttctttctttctttctttctttctttctccttccttcc

SEQ ID NO: 51 - DNA, 78 bp, unidentified
  misc_feature 1..78: note = Description of Unidentified: Illustrative oligonucleotide
  source 1..78: mol_type = unassigned DNA
tttctttctttcttttttctttctttctttctttctttctttctttctttctttctttctttctttctccttccttcc

SEQ ID NO: 52 - DNA, 80 bp, unidentified
  misc_feature 1..80: note = Description of Unidentified: Illustrative oligonucleotide
  source 1..80: mol_type = unassigned DNA
tttctttctttcttttttctctttctttctttctttctttctttctttctttctttctttctttctttctccttccttcc